European Patent Application EP 4 289 277 A1, published December 13, 2023. Title: Method for producing natural cheese. Applicant: AMANO ENZYME INC. The sequence listing filed with the application follows.

SEQUENCE LISTING (15 sequences)

SEQ ID NO: 1 - protein, 549 aa, Artificial Sequence
  P261A mutant of lipase LIP1 derived from Candida cylindracea including signal peptide
MELALALSLIASVAAAPTATLANGDTITGLNAIINEAFLGIPFAEPPVGNLRFKDPVPYSGSLDGQKFTSYGPSCMQQNPEGTYEENLPKAALDLVMQSKVFEAVSPSSEDCLTINVVRPPGTKAGANLPVMLWIFGGGFEVGGTSTFPPAQMITKSIAMGKPIIHVSVNYRVSSWGFLAGDEIKAEGSANAGLKDQRLGMQWVADNIAAFGGDPTKVTIFGESAGSMSVMCHILWNDGDNTYKGKPLFRAGIMQSGAMVASDAVDGIYGNEIFDLLASNAGCGSASDKLACLRGVSSDTLEDATNNTPGFLAYSSLRLSYLPRPDGVNITDDMYALVREGKYANIPVIIGDQNDEGTFFGTSSLNVTTDAQAREYFKQSFVHASDAEIDTLMTAYPGDITQGSPFDTGILNALTPQFKRISAVLGDLGFTLARRYFLNHYTGGTKYSFLSKQLSGLPVLGTFHSNDIVFQDYLLGSGSLIYNNAFIAFATDLDPNTAGLLVKWPEYTSSSQSGNNLMMINALGLYTGKDNFRTAGYDALFSNPPSFFV

SEQ ID NO: 2 - protein, 549 aa, Artificial Sequence
  P261F mutant of lipase LIP1 derived from Candida cylindracea including signal peptide
MELALALSLIASVAAAPTATLANGDTITGLNAIINEAFLGIPFAEPPVGNLRFKDPVPYSGSLDGQKFTSYGPSCMQQNPEGTYEENLPKAALDLVMQSKVFEAVSPSSEDCLTINVVRPPGTKAGANLPVMLWIFGGGFEVGGTSTFPPAQMITKSIAMGKPIIHVSVNYRVSSWGFLAGDEIKAEGSANAGLKDQRLGMQWVADNIAAFGGDPTKVTIFGESAGSMSVMCHILWNDGDNTYKGKPLFRAGIMQSGAMVFSDAVDGIYGNEIFDLLASNAGCGSASDKLACLRGVSSDTLEDATNNTPGFLAYSSLRLSYLPRPDGVNITDDMYALVREGKYANIPVIIGDQNDEGTFFGTSSLNVTTDAQAREYFKQSFVHASDAEIDTLMTAYPGDITQGSPFDTGILNALTPQFKRISAVLGDLGFTLARRYFLNHYTGGTKYSFLSKQLSGLPVLGTFHSNDIVFQDYLLGSGSLIYNNAFIAFATDLDPNTAGLLVKWPEYTSSSQSGNNLMMINALGLYTGKDNFRTAGYDALFSNPPSFFV

SEQ ID NO: 3 - protein, 549 aa, Artificial Sequence
  P261L mutant of lipase LIP1 derived from Candida cylindracea including signal peptide
MELALALSLIASVAAAPTATLANGDTITGLNAIINEAFLGIPFAEPPVGNLRFKDPVPYSGSLDGQKFTSYGPSCMQQNPEGTYEENLPKAALDLVMQSKVFEAVSPSSEDCLTINVVRPPGTKAGANLPVMLWIFGGGFEVGGTSTFPPAQMITKSIAMGKPIIHVSVNYRVSSWGFLAGDEIKAEGSANAGLKDQRLGMQWVADNIAAFGGDPTKVTIFGESAGSMSVMCHILWNDGDNTYKGKPLFRAGIMQSGAMVLSDAVDGIYGNEIFDLLASNAGCGSASDKLACLRGVSSDTLEDATNNTPGFLAYSSLRLSYLPRPDGVNITDDMYALVREGKYANIPVIIGDQNDEGTFFGTSSLNVTTDAQAREYFKQSFVHASDAEIDTLMTAYPGDITQGSPFDTGILNALTPQFKRISAVLGDLGFTLARRYFLNHYTGGTKYSFLSKQLSGLPVLGTFHSNDIVFQDYLLGSGSLIYNNAFIAFATDLDPNTAGLLVKWPEYTSSSQSGNNLMMINALGLYTGKDNFRTAGYDALFSNPPSFFV

SEQ ID NO: 4 - protein, 549 aa, Artificial Sequence
  P261S mutant of lipase LIP1 derived from Candida cylindracea including signal peptide
MELALALSLIASVAAAPTATLANGDTITGLNAIINEAFLGIPFAEPPVGNLRFKDPVPYSGSLDGQKFTSYGPSCMQQNPEGTYEENLPKAALDLVMQSKVFEAVSPSSEDCLTINVVRPPGTKAGANLPVMLWIFGGGFEVGGTSTFPPAQMITKSIAMGKPIIHVSVNYRVSSWGFLAGDEIKAEGSANAGLKDQRLGMQWVADNIAAFGGDPTKVTIFGESAGSMSVMCHILWNDGDNTYKGKPLFRAGIMQSGAMVSSDAVDGIYGNEIFDLLASNAGCGSASDKLACLRGVSSDTLEDATNNTPGFLAYSSLRLSYLPRPDGVNITDDMYALVREGKYANIPVIIGDQNDEGTFFGTSSLNVTTDAQAREYFKQSFVHASDAEIDTLMTAYPGDITQGSPFDTGILNALTPQFKRISAVLGDLGFTLARRYFLNHYTGGTKYSFLSKQLSGLPVLGTFHSNDIVFQDYLLGSGSLIYNNAFIAFATDLDPNTAGLLVKWPEYTSSSQSGNNLMMINALGLYTGKDNFRTAGYDALFSNPPSFFV

SEQ ID NO: 5 - protein, 549 aa, Artificial Sequence
  L322W mutant of lipase LIP1 derived from Candida cylindracea including signal peptide
MELALALSLIASVAAAPTATLANGDTITGLNAIINEAFLGIPFAEPPVGNLRFKDPVPYSGSLDGQKFTSYGPSCMQQNPEGTYEENLPKAALDLVMQSKVFEAVSPSSEDCLTINVVRPPGTKAGANLPVMLWIFGGGFEVGGTSTFPPAQMITKSIAMGKPIIHVSVNYRVSSWGFLAGDEIKAEGSANAGLKDQRLGMQWVADNIAAFGGDPTKVTIFGESAGSMSVMCHILWNDGDNTYKGKPLFRAGIMQSGAMVPSDAVDGIYGNEIFDLLASNAGCGSASDKLACLRGVSSDTLEDATNNTPGFLAYSSLRLSYWPRPDGVNITDDMYALVREGKYANIPVIIGDQNDEGTFFGTSSLNVTTDAQAREYFKQSFVHASDAEIDTLMTAYPGDITQGSPFDTGILNALTPQFKRISAVLGDLGFTLARRYFLNHYTGGTKYSFLSKQLSGLPVLGTFHSNDIVFQDYLLGSGSLIYNNAFIAFATDLDPNTAGLLVKWPEYTSSSQSGNNLMMINALGLYTGKDNFRTAGYDALFSNPPSFFV

SEQ ID NO: 6 - protein, 549 aa, Artificial Sequence
  F360L mutant of lipase LIP1 derived from Candida cylindracea including signal peptide
MELALALSLIASVAAAPTATLANGDTITGLNAIINEAFLGIPFAEPPVGNLRFKDPVPYSGSLDGQKFTSYGPSCMQQNPEGTYEENLPKAALDLVMQSKVFEAVSPSSEDCLTINVVRPPGTKAGANLPVMLWIFGGGFEVGGTSTFPPAQMITKSIAMGKPIIHVSVNYRVSSWGFLAGDEIKAEGSANAGLKDQRLGMQWVADNIAAFGGDPTKVTIFGESAGSMSVMCHILWNDGDNTYKGKPLFRAGIMQSGAMVPSDAVDGIYGNEIFDLLASNAGCGSASDKLACLRGVSSDTLEDATNNTPGFLAYSSLRLSYLPRPDGVNITDDMYALVREGKYANIPVIIGDQNDEGTFLGTSSLNVTTDAQAREYFKQSFVHASDAEIDTLMTAYPGDITQGSPFDTGILNALTPQFKRISAVLGDLGFTLARRYFLNHYTGGTKYSFLSKQLSGLPVLGTFHSNDIVFQDYLLGSGSLIYNNAFIAFATDLDPNTAGLLVKWPEYTSSSQSGNNLMMINALGLYTGKDNFRTAGYDALFSNPPSFFV

SEQ ID NO: 7 - protein, 549 aa, Artificial Sequence
  S380I mutant of lipase LIP1 derived from Candida cylindracea including signal peptide
MELALALSLIASVAAAPTATLANGDTITGLNAIINEAFLGIPFAEPPVGNLRFKDPVPYSGSLDGQKFTSYGPSCMQQNPEGTYEENLPKAALDLVMQSKVFEAVSPSSEDCLTINVVRPPGTKAGANLPVMLWIFGGGFEVGGTSTFPPAQMITKSIAMGKPIIHVSVNYRVSSWGFLAGDEIKAEGSANAGLKDQRLGMQWVADNIAAFGGDPTKVTIFGESAGSMSVMCHILWNDGDNTYKGKPLFRAGIMQSGAMVPSDAVDGIYGNEIFDLLASNAGCGSASDKLACLRGVSSDTLEDATNNTPGFLAYSSLRLSYLPRPDGVNITDDMYALVREGKYANIPVIIGDQNDEGTFFGTSSLNVTTDAQAREYFKQIFVHASDAEIDTLMTAYPGDITQGSPFDTGILNALTPQFKRISAVLGDLGFTLARRYFLNHYTGGTKYSFLSKQLSGLPVLGTFHSNDIVFQDYLLGSGSLIYNNAFIAFATDLDPNTAGLLVKWPEYTSSSQSGNNLMMINALGLYTGKDNFRTAGYDALFSNPPSFFV

SEQ ID NO: 8 - protein, 549 aa, Artificial Sequence
  S380L mutant of lipase LIP1 derived from Candida cylindracea including signal peptide
MELALALSLIASVAAAPTATLANGDTITGLNAIINEAFLGIPFAEPPVGNLRFKDPVPYSGSLDGQKFTSYGPSCMQQNPEGTYEENLPKAALDLVMQSKVFEAVSPSSEDCLTINVVRPPGTKAGANLPVMLWIFGGGFEVGGTSTFPPAQMITKSIAMGKPIIHVSVNYRVSSWGFLAGDEIKAEGSANAGLKDQRLGMQWVADNIAAFGGDPTKVTIFGESAGSMSVMCHILWNDGDNTYKGKPLFRAGIMQSGAMVPSDAVDGIYGNEIFDLLASNAGCGSASDKLACLRGVSSDTLEDATNNTPGFLAYSSLRLSYLPRPDGVNITDDMYALVREGKYANIPVIIGDQNDEGTFFGTSSLNVTTDAQAREYFKQLFVHASDAEIDTLMTAYPGDITQGSPFDTGILNALTPQFKRISAVLGDLGFTLARRYFLNHYTGGTKYSFLSKQLSGLPVLGTFHSNDIVFQDYLLGSGSLIYNNAFIAFATDLDPNTAGLLVKWPEYTSSSQSGNNLMMINALGLYTGKDNFRTAGYDALFSNPPSFFV

SEQ ID NO: 9 - protein, 549 aa, Artificial Sequence
  L425W mutant of lipase LIP1 derived from Candida cylindracea including signal peptide
MELALALSLIASVAAAPTATLANGDTITGLNAIINEAFLGIPFAEPPVGNLRFKDPVPYSGSLDGQKFTSYGPSCMQQNPEGTYEENLPKAALDLVMQSKVFEAVSPSSEDCLTINVVRPPGTKAGANLPVMLWIFGGGFEVGGTSTFPPAQMITKSIAMGKPIIHVSVNYRVSSWGFLAGDEIKAEGSANAGLKDQRLGMQWVADNIAAFGGDPTKVTIFGESAGSMSVMCHILWNDGDNTYKGKPLFRAGIMQSGAMVPSDAVDGIYGNEIFDLLASNAGCGSASDKLACLRGVSSDTLEDATNNTPGFLAYSSLRLSYLPRPDGVNITDDMYALVREGKYANIPVIIGDQNDEGTFFGTSSLNVTTDAQAREYFKQSFVHASDAEIDTLMTAYPGDITQGSPFDTGILNALTPQFKRISAVWGDLGFTLARRYFLNHYTGGTKYSFLSKQLSGLPVLGTFHSNDIVFQDYLLGSGSLIYNNAFIAFATDLDPNTAGLLVKWPEYTSSSQSGNNLMMINALGLYTGKDNFRTAGYDALFSNPPSFFV

SEQ ID NO: 10 - protein, 549 aa, Artificial Sequence
  L428F mutant of lipase LIP1 derived from Candida cylindracea including signal peptide
MELALALSLIASVAAAPTATLANGDTITGLNAIINEAFLGIPFAEPPVGNLRFKDPVPYSGSLDGQKFTSYGPSCMQQNPEGTYEENLPKAALDLVMQSKVFEAVSPSSEDCLTINVVRPPGTKAGANLPVMLWIFGGGFEVGGTSTFPPAQMITKSIAMGKPIIHVSVNYRVSSWGFLAGDEIKAEGSANAGLKDQRLGMQWVADNIAAFGGDPTKVTIFGESAGSMSVMCHILWNDGDNTYKGKPLFRAGIMQSGAMVPSDAVDGIYGNEIFDLLASNAGCGSASDKLACLRGVSSDTLEDATNNTPGFLAYSSLRLSYLPRPDGVNITDDMYALVREGKYANIPVIIGDQNDEGTFFGTSSLNVTTDAQAREYFKQSFVHASDAEIDTLMTAYPGDITQGSPFDTGILNALTPQFKRISAVLGDFGFTLARRYFLNHYTGGTKYSFLSKQLSGLPVLGTFHSNDIVFQDYLLGSGSLIYNNAFIAFATDLDPNTAGLLVKWPEYTSSSQSGNNLMMINALGLYTGKDNFRTAGYDALFSNPPSFFV

SEQ ID NO: 11 - protein, 549 aa, Artificial Sequence
  L428N mutant of lipase LIP1 derived from Candida cylindracea including signal peptide
MELALALSLIASVAAAPTATLANGDTITGLNAIINEAFLGIPFAEPPVGNLRFKDPVPYSGSLDGQKFTSYGPSCMQQNPEGTYEENLPKAALDLVMQSKVFEAVSPSSEDCLTINVVRPPGTKAGANLPVMLWIFGGGFEVGGTSTFPPAQMITKSIAMGKPIIHVSVNYRVSSWGFLAGDEIKAEGSANAGLKDQRLGMQWVADNIAAFGGDPTKVTIFGESAGSMSVMCHILWNDGDNTYKGKPLFRAGIMQSGAMVPSDAVDGIYGNEIFDLLASNAGCGSASDKLACLRGVSSDTLEDATNNTPGFLAYSSLRLSYLPRPDGVNITDDMYALVREGKYANIPVIIGDQNDEGTFFGTSSLNVTTDAQAREYFKQSFVHASDAEIDTLMTAYPGDITQGSPFDTGILNALTPQFKRISAVLGDNGFTLARRYFLNHYTGGTKYSFLSKQLSGLPVLGTFHSNDIVFQDYLLGSGSLIYNNAFIAFATDLDPNTAGLLVKWPEYTSSSQSGNNLMMINALGLYTGKDNFRTAGYDALFSNPPSFFV

SEQ ID NO: 12 - protein, 549 aa, Artificial Sequence
  G429F mutant of lipase LIP1 derived from Candida cylindracea including signal peptide
MELALALSLIASVAAAPTATLANGDTITGLNAIINEAFLGIPFAEPPVGNLRFKDPVPYSGSLDGQKFTSYGPSCMQQNPEGTYEENLPKAALDLVMQSKVFEAVSPSSEDCLTINVVRPPGTKAGANLPVMLWIFGGGFEVGGTSTFPPAQMITKSIAMGKPIIHVSVNYRVSSWGFLAGDEIKAEGSANAGLKDQRLGMQWVADNIAAFGGDPTKVTIFGESAGSMSVMCHILWNDGDNTYKGKPLFRAGIMQSGAMVPSDAVDGIYGNEIFDLLASNAGCGSASDKLACLRGVSSDTLEDATNNTPGFLAYSSLRLSYLPRPDGVNITDDMYALVREGKYANIPVIIGDQNDEGTFFGTSSLNVTTDAQAREYFKQSFVHASDAEIDTLMTAYPGDITQGSPFDTGILNALTPQFKRISAVLGDLFFTLARRYFLNHYTGGTKYSFLSKQLSGLPVLGTFHSNDIVFQDYLLGSGSLIYNNAFIAFATDLDPNTAGLLVKWPEYTSSSQSGNNLMMINALGLYTGKDNFRTAGYDALFSNPPSFFV

SEQ ID NO: 13 - protein, 549 aa, Artificial Sequence
  G429M mutant of lipase LIP1 derived from Candida cylindracea including signal peptide
MELALALSLIASVAAAPTATLANGDTITGLNAIINEAFLGIPFAEPPVGNLRFKDPVPYSGSLDGQKFTSYGPSCMQQNPEGTYEENLPKAALDLVMQSKVFEAVSPSSEDCLTINVVRPPGTKAGANLPVMLWIFGGGFEVGGTSTFPPAQMITKSIAMGKPIIHVSVNYRVSSWGFLAGDEIKAEGSANAGLKDQRLGMQWVADNIAAFGGDPTKVTIFGESAGSMSVMCHILWNDGDNTYKGKPLFRAGIMQSGAMVPSDAVDGIYGNEIFDLLASNAGCGSASDKLACLRGVSSDTLEDATNNTPGFLAYSSLRLSYLPRPDGVNITDDMYALVREGKYANIPVIIGDQNDEGTFFGTSSLNVTTDAQAREYFKQSFVHASDAEIDTLMTAYPGDITQGSPFDTGILNALTPQFKRISAVLGDLMFTLARRYFLNHYTGGTKYSFLSKQLSGLPVLGTFHSNDIVFQDYLLGSGSLIYNNAFIAFATDLDPNTAGLLVKWPEYTSSSQSGNNLMMINALGLYTGKDNFRTAGYDALFSNPPSFFV

SEQ ID NO: 14 - protein, 549 aa, Artificial Sequence
  G429I mutant of lipase LIP1 derived from Candida cylindracea including signal peptide
MELALALSLIASVAAAPTATLANGDTITGLNAIINEAFLGIPFAEPPVGNLRFKDPVPYSGSLDGQKFTSYGPSCMQQNPEGTYEENLPKAALDLVMQSKVFEAVSPSSEDCLTINVVRPPGTKAGANLPVMLWIFGGGFEVGGTSTFPPAQMITKSIAMGKPIIHVSVNYRVSSWGFLAGDEIKAEGSANAGLKDQRLGMQWVADNIAAFGGDPTKVTIFGESAGSMSVMCHILWNDGDNTYKGKPLFRAGIMQSGAMVPSDAVDGIYGNEIFDLLASNAGCGSASDKLACLRGVSSDTLEDATNNTPGFLAYSSLRLSYLPRPDGVNITDDMYALVREGKYANIPVIIGDQNDEGTFFGTSSLNVTTDAQAREYFKQSFVHASDAEIDTLMTAYPGDITQGSPFDTGILNALTPQFKRISAVLGDLIFTLARRYFLNHYTGGTKYSFLSKQLSGLPVLGTFHSNDIVFQDYLLGSGSLIYNNAFIAFATDLDPNTAGLLVKWPEYTSSSQSGNNLMMINALGLYTGKDNFRTAGYDALFSNPPSFFV

SEQ ID NO: 15 - protein, 549 aa, Artificial Sequence
  V549F mutant of lipase LIP1 derived from Candida cylindracea including signal peptide
MELALALSLIASVAAAPTATLANGDTITGLNAIINEAFLGIPFAEPPVGNLRFKDPVPYSGSLDGQKFTSYGPSCMQQNPEGTYEENLPKAALDLVMQSKVFEAVSPSSEDCLTINVVRPPGTKAGANLPVMLWIFGGGFEVGGTSTFPPAQMITKSIAMGKPIIHVSVNYRVSSWGFLAGDEIKAEGSANAGLKDQRLGMQWVADNIAAFGGDPTKVTIFGESAGSMSVMCHILWNDGDNTYKGKPLFRAGIMQSGAMVPSDAVDGIYGNEIFDLLASNAGCGSASDKLACLRGVSSDTLEDATNNTPGFLAYSSLRLSYLPRPDGVNITDDMYALVREGKYANIPVIIGDQNDEGTFFGTSSLNVTTDAQAREYFKQSFVHASDAEIDTLMTAYPGDITQGSPFDTGILNALTPQFKRISAVLGDLGFTLARRYFLNHYTGGTKYSFLSKQLSGLPVLGTFHSNDIVFQDYLLGSGSLIYNNAFIAFATDLDPNTAGLLVKWPEYTSSSQSGNNLMMINALGLYTGKDNFRTAGYDALFSNPPSFFF